European Patent Application EP 4 570 912 A1, published June 18, 2025. Title: METHOD FOR PREPARING LINEAR CLOSED DNA AND PLASMID FOR USE IN THE METHOD. Applicant: Jiangsu GenScript Probio Biotech Co., Ltd. The sequence listing filed with the application follows.

SEQUENCE LISTING (2 sequences)

SEQ ID NO: 1 - DNA, 56 bp, synthetic construct
  source 1..56: mol_type = other DNA; note = TelRL
tatcagcacacaattgcccattatacgcgcgtataatggactattgtgtgctgata

SEQ ID NO: 2 - DNA, 2017 bp, synthetic construct
  source 1..2017: mol_type = other DNA; note = CFL universal
tcgcgcgtttcggtgatgacggtgaaaacctctgacacataagcttgcatgcaggcctctgcagtcgacgggcccgggatcctatcagcacacaattgcccattatacgcgcgtataatggactattgtgtgctgatatatcagcacacaattgcccattatacgcgcgtataatggactattgtgtgctgatagatatctagatgcattcgcgaggtaccgagctcgaattcgcagctcccggacgtcattgtcgatatcattgtcacatgtgagcaaaaggccagcaaaaggccaggaaccgtaaaaaggccgcgttgctggcgtttttccataggctccgcccccctgacgagcatcacaaaaatcgacgctcaagtcagaggtggcgaaacccgacaggactataaagataccaggcgtttccccctggaagctccctcgtgcgctctcctgttccgaccctgccgcttaccggatacctgtccgcctttctcccttcgggaagcgtggcgctttctcatagctcacgctgtaggtatctcagttcggtgtaggtcgttcgctccaagctgggctgtgtgcacgaaccccccgttcagcccgaccgctgcgccttatccggtaactatcgtcttgagtccaacccggtaagacacgacttatcgccactggcagcagccactggtaacaggattagcagagcgaggtatgtaggcggtgctacagagttcttgaagtggtggcctaactacggctacactagaagaacagtatttggtatctgcgctctgctgaagccagttaccttcggaaaaagagttggtagctcttgatccggcaaacaaaccaccgctggtagcggtggtttttttgtttgcaagcagcagattacgcgcagaaaaaaaggatctcaagaagatcctttgatcttttctacggggtctgacgctcagtggaacgaaaactcacgttaagggattttggtcatgagattatcaaaaaggatcttcacctagatccttttaaattaaaaatgaagttttaaatcaagcccaatctgaataatgttacaaccaattaaccaattctgattagaaaaactcatcgagcatcaaatgaaactgcaatttattcatatcaggattatcaataccatatttttgaaaaagccgtttctgtaatgaaggagaaaactcaccgaggcagttccataggatggcaagatcctggtatcggtctgcgattccgactcgtccaacatcaatacaacctattaatttcccctcgtcaaaaataaggttatcaagtgagaaatcaccatgagtgacgactgaatccggtgagaatggcaaaagtttatgcatttctttccagacttgttcaacaggccagccattacgctcgtcatcaaaatcactcgcatcaaccaaaccgttattcattcgtgattgcgcctgagcgagacgaaatacgcgatcgctgttaaaaggacaattacaaacaggaatcgaatgcaaccggcgcaggaacactgccagcgcatcaacaatattttcacctgaatcaggatattcttctaatacctggaatgctgtttttccggggatcgcagtggtgagtaaccatgcatcatcaggagtacggataaaatgcttgatggtcggaagaggcataaattccgtcagccagtttagtctgaccatctcatctgtaacatcattggcaacgctacctttgccatgtttcagaaacaactctggcgcatcgggcttcccatacaagcgatagattgtcgcacctgattgcccgacattatcgcgagcccatttatacccatataaatcagcatccatgttggaatttaatcgcggcctcgacgtttcccgttgaatatggctcataacaccccttgtattactgtttatgtaagcagacagttttattgttcatgatgatatatttttatcttgtgcaatgtaacatcagagattttgagacacgggccagagctgca